European Patent Specification EP 3 710 015 B1, published January 17, 2024. Title: Use of SRSF3 agents for the treatment and/or prevention of neurological conditions, cancer, bacterial infections or viral infections. Applicant: Universite Laval. The sequence listing filed with the application follows.

SEQUENCE LISTING (20 sequences)

SEQ ID NO: 1 - DNA, 5306 bp, Artificial Sequence
  Flag/EGFP tagged murine Rpl10a construction under control of the CD11b promoter, I: Intervening sequence (IVS); II: SV40 polyA
gggccctccagggttcaagtgattctgctgcctcagcctcccaggtgggattacaggtgcctgccaccacgcctggctaatttttttgtctttttagtaaagatgaggtttcaccatgttgggcaggctggtttcaattgctgacctcaagtgagccaccccgcctcagcctcccaaaatgctaggattacaggcatgagccaccgcacccagccaagtttgtacatatatttttgactacacttcttaactattcttaggataaattactagaagtgaaaattcttgggtgaagagcttgaggcctttacacacacacacacacacacacacaaaaataggctggatgcagtggctcacacctgtaatctcagcagtttgggaggctgaggaaggaggatcacttgagtccaggaggttgagaatagcctgaacaacatagcaagatcttgtctctacaaaaaatttaaaaaaaattagctggccatggcagcatgtgcctgtagtaccagctactcggaaggctgaggtaggaggatcgcttgagcccaggaggttgattgaagctgcagtgagctgtgattacaccactgcactccagcctgggcaacagagctagactctgtctctaaaaaaagcacaaaataatatttaaaaagcaccaggtatgcctgtacttgagttgtctttgttgatggctacaaatgaggacagctctggctgaagggcgcttccatttccatgggctgaaggagggacattttgcaaagtgtgttttcaggaagacacagagttttacctcctacacttgtttgatctgtattaatgtttgcttatttatttatttaattttttttttgagacagagtctcactctgtcacctgggctggagtgcagtggcattattgaggctcattgcagtctcagactcctgagctcaaacaatcctcctgcctcagcctctggagtagctaggactacaggcatgtgccaccatgcctggctaattttttaaatgtatttttttgtagagtcggggtctccctatgttgcccaggctggagtgcagtggtgtgatcctagctcactgcagcctggacctcgggctcaagtaattctcacacctcagcctgtccagtagcaggggctacaggcgcgcaccaccatgcccagctaattaaaaatatttttttgtagagacagggtctctctatgttgcccaggctggtttcaaactcccaggctcaagcaatcctcctgccttggcctcccaaagtgctggcattacaggcgtgagccactgcgcctggcccgtattaatgtttagaacacgaattccaggaggcaggctaagtctgttcagcttgttcatatgcttgggccaacccaagaaacaagtgggtgacaaatggcaccttttggatagtggtattgactttgaaagtttgggtcaggaagctggggaggaagggtgggcaggctgtgggcagtcctgggcggaagaccaggcagggctatgtgctcactgagcctccgccctcttcctttgaatctctgatagacttctgcctcctacttctccttttctgcccttctttgctttggtggcttccttgtggttcctcagtggtgcctgcaacccctggttcacctccttccaggttctggctccttccagccgtcgacggtatcgataagcttgatatctaagtatcaaggttacaagacaggtttaaggagaccaatagaaactgggcttgtcgagacagagaagactcttgcgtttctgataggcacctattggtcttactgacatccactttctttctctccacaggaattccctgcaggaggcagcatggactacaaagacgacgacgacaaggtgagcaagggcgaggagctgttcaccggggtggtgcccatcctggtcgagctggacggcgacgtaaacggccacaagttcagcgtgtccggcgagggcgagggcgatgccacctacggcaagctgaccctgaagttcatctgcaccaccggcaagctgcccgtgccctggcccaccctcgtgaccaccctgacctacggcgtgcagtgcttcagccgctaccccgaccacatgaagcagcacgacttcttcaagtccgccatgcccgaaggctacgtccaggagcgcaccatcttcttcaaggacgacggcaactacaagacccgcgccgaggtgaagttcgagggcgacaccctggtgaaccgcatcgagctgaagggcatcgacttcaaggaggacggcaacatcctggggcacaagctggagtacaactacaacagccacaacgtctatatcatggccgacaagcagaagaacggcatcaaggtgaacttcaagatccgccacaacatcgaggacggcagcgtgcagctcgccgaccactaccagcagaacacccccatcggcgacggccccgtgctgctgcccgacaaccactacctgagcacccagtccgccctgagcaaagaccccaacgagaagcgcgatcacatggtcctgctggagttcgtgaccgccgccgggatcactctcggcatggacgagctgtacaagtaaggatcccggccgcaaactgcagcgcctctccggcttggctgagcgcggaacgtgcccgtaacgggcaactctcgcgagaacgcgggctctatttgagcgcatgcgcaaagcgctctgccttctttccggtttccgcggcagccgcagccatgaggtaagttgttatcgtggcgctatccgccgccatccgtgcacccacacgcccgcggacgccccgcggcccgtctcggaggctctcccggcgactgccccgcgtcgcgagcctttccccagcgtgccgtgggcctgtcatcgggcccggggtgcagcatggccggccccgaacgccttcgcttctccccaacagcagcaaagtctcacgcgacaccctgtacgaggcggtgcgggaagtcctgcacgggaaccagcgcaagcgccgcaagtgagcgcgggcctccctcccggggcagggcgagcatccccggccatggcgaccctggctcacagctcccctctcgctcaggtttctggagacggtggagctgcagatcagcctgaagaactacgaccctcagaaggacaaacgtttctcgggcaccgtcaggttggcaccgctctaaccccacccagccctcagtgttcccgtgtggcctggccgcgccctaggcgggcacggggacactgacgtgccagggtagttcaggagccctgctgcaggcaggcaggctggacggacccccaccctgggtcttaaaacaagaggggaggcgtggggaggcctcggccgagcccgccgcctagcctgagaagccaggctagtgttgcccagagctccgggtaaggcttgccgctccctgccatgcgttcagatctagcgggatggccagcgccgaccatgacctgttctgttttctcccctcccaaacgcaggctcaagtccaccccacgccccaagttctcggtgtgcgttctgggggaccagcagcactgtgatgaagccaaggccgtggatatcccccacatggacatcgaggcgctcaagaagcttaacaaaaacaagaagttggtcaagaagctgggtaggtggggctcactagggctgaacacaacccatgaccccctgcccaggagtggcagcacacattgggcttcacaaccagttagaaaatgccccacaggctggtctgatactcccctctcgccagtgtgtgcagttgactcatagccagctattggtttgggtttcaagtcttttcagttaacaacctatcgagggaggggtcacaagtgtctcccacgtgttagcctccatggtagcccctgtctccgcatacattttgggaatagttatccactgtgagctaggcagttgtcatgcctgcttttatagatagaaggtttctccatctgtcttaagatttggagtaatactgagtcttactgatgttgccagcctggggtctaaggttatcctctagaagtgctcaggactgtgccctgtcactgagctgtgttctcaggtgacattatggttcccaggcctgcttgaggcttctcagatagctggccttggtccacctttgacagataatgagacagcttttttcttaagattttattttatgtatatgagcaggctgatgagagcctcagatcccattacaggtggctgtgagccaccatgtggctgctggaaattgaactcaggacctctggaaggcagcactcttaactgctgagccatctctccagtccatagtttgaggcaatttaaatgcaggcttacagtgaatccaaggggtgggggccatcacagcccctcagttctatgcagcacaccagggattgtgggacatcctggtctaagacctctgtgaggacttgagggtggagctactcagcagtcatgggtctgaggaggcaacttggccttctcgttgtaaaggatgggttggttgtttaaaatgttttgttttgtttttttttttttttggtggtttttgtttgtttggttggtttttttggtttttttggtttttttttttttttttggctcaatcctgagtgtctgtgtcttctagctaagaagtacgatgcctttttggcctctgagtctctgattaagcagatcccacgtatcctgggcccaggcctaaacaaggctggcaagttcccctccctgctgacacacaatgaaaacatggtggccaaagtggatgaggtgaaatcgacaatcaagttccagatgaagaaggtcagtctgggcggtgtgtggtggggaaaccagaaagagctaggtctgggtgccttagccctgggttaagccttttcactgggggaaagggtacatgctagcttagcctggtgaccttttctgtccatgcaggtgctgtgtttggccgtcgctgttggccacgtgaagatgaccgatgatgagctagtctacaacattcatctggctgtcaatttcttggtgtccttgcttaagaaaaactggcaaaacgtgcgggctctgtacatcaagagcaccatgggcaagccccagcgtctgtattaggatgctccaataaacctcactgctgccactcaggcggccgcaccgcggttgatgagtttggacaaaccacaactagaatgcagtgaaaaaaatgctttatttgtgaaatttgtgatgctattgctttatttgtaaccattataagctgcaataaacaagttccgcgg

SEQ ID NO: 2 - DNA, 86 bp, Artificial Sequence
  pGL3-promoter- Saa3-3'UTR-wt
gttttctcttcctgttgttcccagtcatgctgccccccgagaagaggagcaactactgggttgagatattttctaaaatctggatc

SEQ ID NO: 3 - DNA, 168 bp, Artificial Sequence
  pGL3-promoter-SCRAMBLE
ggatatcttttacccatacgatgttcctgactatgcgggctatccctatgacgtcccggactatgcaggatcctatccatatgacgttccagattacgctgctcagatcgataagcttaccatgttccaggcggccgagcgcccccaggagtgggccatggagggccc

SEQ ID NO: 4 - DNA, 87 bp, Artificial Sequence
  Saa3-3'UTR deletion of segment C
gttttctcttcctgttgttcccagtcatgctgccccccgagaagaggagcaactactgggttgagatattttctaaaatctggatcc

SEQ ID NO: 5 - DNA, 45 bp, Artificial Sequence
  Saa3-3'UTR deletion of segment B+C
gttttctcttcctgttgttcccagtcatgctgccccccgtctaga

SEQ ID NO: 6 - DNA, 89 bp, Artificial Sequence
  Saa3-3'UTR deletion of segment A
agaagaggagcaactactgggttgagatattttctaaaatctggatccctaaacatcccaatgtgctgaataaatacttgtgaaatgca

SEQ ID NO: 7 - DNA, 69 bp, Artificial Sequence
  Saa3-3'UTR deletion of segment B
gttttctcttcctgttgttcccagtcatgctgccccccgaatgtgctgaataaatacttgtgaaatgca

SEQ ID NO: 8 - RNA, 19 nt, Artificial Sequence
  siRNA targeting SRSF3 - ON-TARGETplus SMARTpool siRNA J-059214-09, Srsf3
gaaaggcaccugagaauau

SEQ ID NO: 9 - RNA, 19 nt, Artificial Sequence
  siRNA targeting SRSF3 - ON-TARGETplus SMARTpool siRNA J-059214-10, Srsf3
ccagaugagauuuagguau

SEQ ID NO: 10 - RNA, 19 nt, Artificial Sequence
  siRNA targeting SRSF3 - ON-TARGETplus SMARTpool siRNA J-059214-11, Srsf3
cuagcauaauuguguagua

SEQ ID NO: 11 - RNA, 19 nt, Artificial Sequence
  siRNA targeting SRSF3 - ON-TARGETplus SMARTpool siRNA J-059214-12, Srsf3
cuagaagguuccaacauga

SEQ ID NO: 12 - protein, 164 aa, Mus musculus
MHRDSCPLDCKVYVGNLGNNGNKTELERAFGYYGPLRSVWVARNPPGFAFVEFEDPRDAADAVRELDGRTLCGCRVRVELSNGEKRSRNRGPPPSWGRRPRDDYRRRSPPPRRRSPRRRSFSRSRSRSLSRDRRRERSLSRERNHKPSRSFSRSRSRSRSNERK

SEQ ID NO: 13 - protein, 73 aa, Mus musculus
KVYVGNLGNNGNKTELERAFGYYGPLRSVWVARNPPGFAFVEFEDPRDAADAVRELDGRTLCGCRVRVELSNG

SEQ ID NO: 14 - protein, 79 aa, Mus musculus
RSRNRGPPPSWGRRPRDDYRRRSPPPRRRSPRRRSFSRSRSRSLSRDRRRERSLSRERNHKPSRSFSRSRSRSRSNERK

SEQ ID NO: 15 - DNA, 25 bp, Artificial Sequence
  Antisense
ccaagggacaggaatcacgatgcat

SEQ ID NO: 16 - DNA, 84 bp, Mus musculus
ggtgggcctgtcggagcgttaggatttgagcttgggccttttgaacccaggatctcgaaatgcatcgtgattcctgtcccttgg

SEQ ID NO: 17 - DNA, 25 bp, Artificial Sequence
  Antisense
ccaatggacaggaatcacgatgcat

SEQ ID NO: 18 - DNA, 56 bp, Homo sapiens
gccgccgcattttttaaccctagatctcgaaatgcatcgtgattcctgtccattgg

SEQ ID NO: 19 - DNA, 720 bp, Homo sapiens
tttccaggtcacctgaccggtctcctttgctgtcggcgccaagtcctgcaagtttgcttgagagacgagaaaccagcaagagttgggcaaactttccaaaccaggcttttccttcagtgtggaatctaggcggccacagtctggtgccagctgggtcacaaacagctccgtgacctgtttgtaaacgcgatgctcttagttccagactaaccgctcacaagggtgaagcacttaattaattcatctcttaatcttgttaggggccaacggctcctattagtgtttgagcgtgacggcgacggtgctgtttatgaagccctagcctatttggaggtgaggaagaggagtctgtgggtaacctggaggtcgacagaccgggaggaacgctcgagggagcaccaggcctgttacaacgagcgcgcgccgacgcacgtctccacccacccggcgcaaccgccagagcgcgctcccagcaaccgcggctctcgctgcgtttgtagccatacgtcacggcctcttctgcttctcattgggggagcccgtccaatcatgtgattccagtatggcgtataaataaaggcgaggagaaggcggtggtccgccatttcgtggacgccgggtgagtgagagagttggttggtgttgggccggaggaaagcgggaagactcatcggagcgtgtggatttgagccgccgcattttttaaccctagatctcgaa

SEQ ID NO: 20 - protein, 22 aa, Artificial Sequence
  Fragment
GNNGNKTELERAFGYYGPLRSV